European Patent Specification EP 3 315 514 B1, published June 18, 2025. Title: Blood brain barrier shuttles. Applicant: F. Hoffmann-La Roche AG. The sequence listing filed with the application follows.

SEQUENCE LISTING (17 sequences)

SEQ ID NO: 1 - protein, 959 aa, Artificial Sequence
  Fusion polypeptide
MGWSCIILFLVATATGVHSQVELVESGGGLVQPGGSLRLSCAASGFTFSSYAMSWVRQAPGKGLEWVSAINASGTRTYYADSVKGRFTISRDNSKNTLYLQMNSLRAEDTAVYYCARGKGNTHKPYGYVRYFDVWGQGTLVTVSSASTKGPSVFPLAPSSKSTSGGTAALGCLVKDYFPEPVTVSWNSGALTSGVHTFPAVLQSSGLYSLSSVVTVPSSSLGTQTYICNVNHKPSNTKVDKKVEPKSCDKTHTCPPCPAPELLGGPSVFLFPPKPKDTLMISRTPEVTCVVVDVSHEDPEVKFNWYVDGVEVHNAKTKPREEQYNSTYRVVSVLTVLHQDWLNGKEYKCKVSNKALPAPIEKTISKAKGQPREPQVYTLPPSRDELTKNQVSLTCLVKGFYPSDIAVEWESNGQPENNYKTTPPVLDSDGSFFLYSKLTVDKSRWQQGNVFSCSVMHEALHNHYTQKSLSLSPGGGSGGGGSGGGGSGGGGSDIQMTQSPASLSASLEEIVTITCQASQDIGNWLAWYQQKPGKSPQLLIYGATSLADGVPSRFSGSRSGTQFSLKISRVQVEDIGIYYCLQAYNTPWTFGGGTKVEIKRTVAAPSVFIFPPSDEQLKSGTASVVCLLNNFYPREAKVQWKVDNALQSGNSQESVTEQDSKDSTYSLSSTLTLSKADYEKHKVYACEVTHQGLSSPVTKSFNRGECGGGGSGGGGSGGGGSGGGGSGGGGSGGGGSGGEVQLVESGGGLVQPGNSLTLSCVASGFTFSNYGMHWIRQAPKKGLEWIAMIYYDSSKMNYADTVKGRFTISRDNSKNTLYLEMNSLRSEDTAMYYCAVPTSHYVVDVWGQGVSVTVSSASTKGPSVFPLAPSSKSTSGGTAALGCLVKDYFPEPVTVSWNSGALTSGVHTFPAVLQSSGLYSLSSVVTVPSSSLGTQTYICNVNHKPSNTKVDKKVEPKSC

SEQ ID NO: 2 - protein, 234 aa, Artificial Sequence
  Light chain construct
MGWSCIILFLVATATGVHSDIVLTQSPATLSLSPGERATLSCRASQSVSSSYLAWYQQKPGQAPRLLIYGASSRATGVPARFSGSGSGTDFTLTISSLEPEDFATYYCLQIYNMPITFGQGTKVEIKRTVAAPSVFIFPPSDEQLKSGTASVVCLLNNFYPREAKVQWKVDNALQSGNSQESVTEQDSKDSTYSLSSTLTLSKADYEKHKVYACEVTHQGLSSPVTKSFNRGEC

SEQ ID NO: 3 - protein, 959 aa, Artificial Sequence
  Fusion polypeptide
MGWSCIILFLVATATGVHSQVELVESGGGLVQPGGSLRLSCAASGFTFSSYAMSWVRQAPGKGLEWVSAINASGTRTYYADSVKGRFTISRDNSKNTLYLQMNSLRAEDTAVYYCARGKGNTHKPYGYVRYFDVWGQGTLVTVSSASTKGPSVFPLAPSSKSTSGGTAALGCLVKDYFPEPVTVSWNSGALTSGVHTFPAVLQSSGLYSLSSVVTVPSSSLGTQTYICNVNHKPSNTKVDKKVEPKSCDKTHTCPPCPAPELLGGPSVFLFPPKPKDTLMISRTPEVTCVVVDVSHEDPEVKFNWYVDGVEVHNAKTKPREEQYNSTYRVVSVLTVLHQDWLNGKEYKCKVSNKALPAPIEKTISKAKGQPREPQVYTLPPCRDELTKNQVSLWCLVKGFYPSDIAVEWESNGQPENNYKTTPPVLDSDGSFFLYSKLTVDKSRWQQGNVFSCSVMHEALHNHYTQKSLSLSPGGGSGGGGSGGGGSGGGGSDIQMTQSPASLSASLEEIVTITCQASQDIGNWLAWYQQKPGKSPQLLIYGATSLADGVPSRFSGSRSGTQFSLKISRVQVEDIGIYYCLQAYNTPWTFGGGTKVEIKRTVAAPSVFIFPPSDEQLKSGTASVVCLLNNFYPREAKVQWKVDNALQSGNSQESVTEQDSKDSTYSLSSTLTLSKADYEKHKVYACEVTHQGLSSPVTKSFNRGECGGGGSGGGGSGGGGSGGGGSGGGGSGGGGSGGEVQLVESGGGLVQPGNSLTLSCVASGFTFSNYGMHWIRQAPKKGLEWIAMIYYDSSKMNYADTVKGRFTISRDNSKNTLYLEMNSLRSEDTAMYYCAVPTSHYVVDVWGQGVSVTVSSASTKGPSVFPLAPSSKSTSGGTAALGCLVKDYFPEPVTVSWNSGALTSGVHTFPAVLQSSGLYSLSSVVTVPSSSLGTQTYICNVNHKPSNTKVDKKVEPKSC

SEQ ID NO: 4 - protein, 475 aa, Artificial Sequence
  Fusion polypeptide
MGWSCIILFLVATATGVHSQVELVESGGGLVQPGGSLRLSCAASGFTFSSYAMSWVRQAPGKGLEWVSAINASGTRTYYADSVKGRFTISRDNSKNTLYLQMNSLRAEDTAVYYCARGKGNTHKPYGYVRYFDVWGQGTLVTVSSASTKGPSVFPLAPSSKSTSGGTAALGCLVKDYFPEPVTVSWNSGALTSGVHTFPAVLQSSGLYSLSSVVTVPSSSLGTQTYICNVNHKPSNTKVDKKVEPKSCDKTHTCPPCPAPELLGGPSVFLFPPKPKDTLMISRTPEVTCVVVDVSHEDPEVKFNWYVDGVEVHNAKTKPREEQYNSTYRVVSVLTVLHQDWLNGKEYKCKVSNKALPAPIEKTISKAKGQPREPQVCTLPPSRDELTKNQVSLSCAVKGFYPSDIAVEWESNGQPENNYKTTPPVLDSDGSFFLVSKLTVDKSRWQQGNVFSCSVMHEALHNHYTQKSLSLSPGK

SEQ ID NO: 5 - protein, 10 aa, Homo sapiens
GFTFSSYAMS

SEQ ID NO: 6 - protein, 17 aa, Homo sapiens
AINASGTRTYYADSVKG

SEQ ID NO: 7 - protein, 17 aa, Homo sapiens
GKGNTHKPYGYVRYFDV

SEQ ID NO: 8 - protein, 12 aa, Homo sapiens
RASQSVSSSYLA

SEQ ID NO: 9 - protein, 7 aa, Homo sapiens
GASSRAT

SEQ ID NO: 10 - protein, 8 aa, Homo sapiens
LQIYNMPI

SEQ ID NO: 11 - protein, 126 aa, Homo sapiens [sequence omitted]

SEQ ID NO: 12 - protein, 110 aa, Homo sapiens
DIVLTQSPATLSLSPGERATLSCRASQSVSSSYLAWYQQKPGQAPRLLIYGASSRATGVPARFSGSGSGTDFTLTISSLEPEDFATYYCLQIYNMPITFGQGTKVEIKRT

SEQ ID NO: 13 - protein, 32 aa, Artificial Sequence
  Peptide linker
GGGGSGGGGSGGGGSGGGGSGGGGSGGGGSGG

SEQ ID NO: 14 - protein, 15 aa, Artificial Sequence
  Epitope mapping peptide
IGQNMVTIVQSNGNL

SEQ ID NO: 15 - protein, 15 aa, Artificial Sequence
  Epitope mapping peptide
NMVTIVQSNGNLDPV

SEQ ID NO: 16 - protein, 15 aa, Artificial Sequence
  Epitope mapping peptide
QSNGNLDPVESPEGY

SEQ ID NO: 17 - protein, 20 aa, Artificial Sequence
  Peptide linker
GGGGSGGGGSGGGGSGGGGS